European Patent Application EP 4 545 643 A1, published April 30, 2025. Title: Plasmids for improved AAV titers and empty full ratios. Applicant: Sartorius Stedim Cellca GmbH. The sequence listing filed with the application follows.

SEQUENCE LISTING (18 sequences)

SEQ ID NO: 1 - DNA, 145 bp, adeno-associated virus 2
  source 1..145: mol_type = other DNA
ttggccactccctctctgcgcgctcgctcgctcactgaggccgggcgaccaaaggtcgcccgacgcccgggctttgcccgggcggcctcagtgagcgagcgagcgcgcagagagggagtggccaactccatcactaggggttcct

SEQ ID NO: 2 - DNA, 145 bp, adeno-associated virus 2
  source 1..145: mol_type = other DNA
aggaacccctagtgatggagttggccactccctctctgcgcgctcgctcgctcactgaggccgggcgaccaaaggtcgcccgacgcccgggctttgcccgggcggcctcagtgagcgagcgagcgcgcagagagggagtggccaa

SEQ ID NO: 3 - DNA, 1944 bp, synthetic construct
  source 1..1944: mol_type = other DNA
ttggccactccctctctgcgcgctcgctcgctcactgaggccgggcgaccaaaggtcgcccgacgcccgggctttgcccgggcggcctcagtgagcgagcgagcgcgcagagagggagtggccaactccatcactaggggttcctgtcgacggatccctgcagcgtctcgcatgctagttattaatagtaatcaattacggggtcattagttcatagcccatatatggagttccgcgttacataacttacggtaaatggcccgcctggctgaccgcccaacgacccccgcccattgacgtcaataatgacgtatgttcccatagtaacgccaatagggactttccattgacgtcaatgggtggagtatttacggtaaactgcccacttggcagtacatcaagtgtatcatatgccaagtacgccccctattgacgtcaatgacggtaaatggcccgcctggcattatgcccagtacatgaccttatgggactttcctacttggcagtacatctacgtattagtcatcgctattaccatggtgatgcggttttggcagtacatcaatgggcgtggatagcggtttgactcacggggatttccaagtctccaccccattgacgtcaatgggagtttgttttggcaccaaaatcaacgggactttccaaaatgtcgtaacaactccgccccattgacgcaaatgggcggtaggcgtgtacggtgggaggtctatataagcagagctggtttagtgaaccgtcagatccgctagcgctaccggtcgccaccatggtgagcaagggcgaggagctgttcaccggggtggtgcccatcctggtcgagctggacggcgacgtaaacggccacaagttcagcgtgtccggcgagggcgagggcgatgccacctacggcaagctgaccctgaagttcatctgcaccaccggcaagctgcccgtgccctggcccaccctcgtgaccaccctgacctacggcgtgcagtgcttcagccgctaccccgaccacatgaagcagcacgacttcttcaagtccgccatgcccgaaggctacgtccaggagcgcaccatcttcttcaaggacgacggcaactacaagacccgcgccgaggtgaagttcgagggcgacaccctggtgaaccgcatcgagctgaagggcatcgacttcaaggaggacggcaacatcctggggcacaagctggagtacaactacaacagccacaacgtctatatcatggccgacaagcagaagaacggcatcaaggtgaacttcaagatccgccacaacatcgaggacggcagcgtgcagctcgccgaccactaccagcagaacacccccatcggcgacggccccgtgctgctgcccgacaaccactacctgagcacccagtccgccctgagcaaagaccccaacgagaagcgcgatcacatggtcctgctggagttcgtgaccgccgccgggatcactctcggcatggatgagctgtataagagcggactgagatccagagcccaggctagcaactctgctgtggacggaacagctggcccaggcagtaccggctccagatgactgatcataatcagccataccacatttgtagaggttttacttgctttaaaaaacctcccacacctccccctgaacctgaaacataaaatgaatgcaattgttgttgttaacttgtttattgcagcttataatggttacaaataaagcaatagcatcacaaatttcacaaataaagcattttttatcgatggtcacccatatgggtaccgagctcaggaacccctagtgatggagttggccactccctctctgcgcgctcgctcgctcactgaggccgggcgaccaaaggtcgcccgacgcccgggctttgcccgggcggcctcagtgagcgagcgagcgcgcagagagggagtggccaa

SEQ ID NO: 4 - DNA, 122 bp, synthetic construct
  source 1..122: mol_type = other DNA
ttggccactccctctctgcgcgctcgctcgctcactgaggccgggcgaccaaaggtcgcccgacgcccgggctttgcccgggcggcctcagtgagcgagcgagcgcgcagagagggagtggt

SEQ ID NO: 5 - DNA, 1924 bp, synthetic construct
  source 1..1924: mol_type = other DNA
ttggccactccctctctgcgcgctcgctcgctcactgaggccgggcgaccaaaggtcgcccgacgcccgggctttgcccgggcggcctcagtgagcgagcgagcgcgcagagagggagtggtgtcgacggatccctgcagcgtctcgcatgctagttattaatagtaatcaattacggggtcattagttcatagcccatatatggagttccgcgttacataacttacggtaaatggcccgcctggctgaccgcccaacgacccccgcccattgacgtcaataatgacgtatgttcccatagtaacgccaatagggactttccattgacgtcaatgggtggagtatttacggtaaactgcccacttggcagtacatcaagtgtatcatatgccaagtacgccccctattgacgtcaatgacggtaaatggcccgcctggcattatgcccagtacatgaccttatgggactttcctacttggcagtacatctacgtattagtcatcgctattaccatggtgatgcggttttggcagtacatcaatgggcgtggatagcggtttgactcacggggatttccaagtctccaccccattgacgtcaatgggagtttgttttggcaccaaaatcaacgggactttccaaaatgtcgtaacaactccgccccattgacgcaaatgggcggtaggcgtgtacggtgggaggtctatataagcagagctggtttagtgaaccgtcagatccgctagcgctaccggtcgccaccatggtgagcaagggcgaggagctgttcaccggggtggtgcccatcctggtcgagctggacggcgacgtaaacggccacaagttcagcgtgtccggcgagggcgagggcgatgccacctacggcaagctgaccctgaagttcatctgcaccaccggcaagctgcccgtgccctggcccaccctcgtgaccaccctgacctacggcgtgcagtgcttcagccgctaccccgaccacatgaagcagcacgacttcttcaagtccgccatgcccgaaggctacgtccaggagcgcaccatcttcttcaaggacgacggcaactacaagacccgcgccgaggtgaagttcgagggcgacaccctggtgaaccgcatcgagctgaagggcatcgacttcaaggaggacggcaacatcctggggcacaagctggagtacaactacaacagccacaacgtctatatcatggccgacaagcagaagaacggcatcaaggtgaacttcaagatccgccacaacatcgaggacggcagcgtgcagctcgccgaccactaccagcagaacacccccatcggcgacggccccgtgctgctgcccgacaaccactacctgagcacccagtccgccctgagcaaagaccccaacgagaagcgcgatcacatggtcctgctggagttcgtgaccgccgccgggatcactctcggcatggatgagctgtataagagcggactgagatccagagcccaggctagcaactctgctgtggacggaacagctggcccaggcagtaccggctccagatgactgatcataatcagccataccacatttgtagaggttttacttgctttaaaaaacctcccacacctccccctgaacctgaaacataaaatgaatgcaattgttgttgttaacttgtttattgcagcttataatggttacaaataaagcaatagcatcacaaatttcacaaataaagcattttttatcgatggtcacccatatgggtaccgagctcaggaacccctagtgatggagttggccactccctctctgcgcgctcgctcgctcactgaggccgggcgaccaaaggtcgcccgacgcccgggctttgcccgggcggcctcagtgagcgagcgagcgcgcagagagggagtggccaagcg

SEQ ID NO: 6 - DNA, 99 bp, synthetic construct
  source 1..99: mol_type = other DNA
ctctgcgtatttctttcttatctagtttccatggctacgtagataagtagcatggcgggttaatcattaactacaatcagtgagcgagcgagcgcgcag

SEQ ID NO: 7 - DNA, 4447 bp, synthetic construct
  source 1..4447: mol_type = other DNA
ggtggagtcgtgacgtgaattacgtcatagggttagggaggtcctgtattagaggtcacgtgagtgttttgcgacattttgcgacaccatgtggtcacgctgggtatttaagcccgagtgagcacgcagggtctccattttgaagcgggaggtttgaacgcgcagccgccatgccggggttttacgagattgtgattaaggtccccagcgaccttgacgagcatctgcccggcatttctgacagctttgtgaactgggtggccgagaaggaatgggagttgccgccagattctgacatggatctgaatctgattgagcaggcacccctgaccgtggccgagaagctgcagcgcgactttctgacggaatggcgccgtgtgagtaaggccccggaggcccttttctttgtgcaatttgagaagggagagagctacttccacatgcacgtgctcgtggaaaccaccggggtgaaatccatggttttgggacgtttcctgagtcagattcgcgaaaaactgattcagagaatttaccgcgggatcgagccgactttgccaaactggttcgcggtcacaaagaccagaaatggcgccggaggcgggaacaaggtggtggatgagtgctacatccccaattacttgctccccaaaacccagcctgagctccagtgggcgtggactaatatggaacagtatttaagcgcctgtttgaatctcacggagcgtaaacggttggtggcgcagcatctgacgcacgtgtcgcagacgcaggagcagaacaaagagaatcagaatcccaattctgatgcgccggtgatcagatcaaaaacttcagccaggtacatggagctggtcgggtggctcgtggacaaggggattacctcggagaagcagtggatccaggaggaccaggcctcatacatctccttcaatgcggcctccaactcgcggtcccaaatcaaggctgccttggacaatgcgggaaagattatgagcctgactaaaaccgcccccgactacctggtgggccagcagcccgtggaggacatttccagcaatcggatttataaaattttggaactaaacgggtacgatccccaatatgcggcttccgtctttctgggatgggccacgaaaaagttcggcaagaggaacaccatctggctgtttgggcctgcaactaccgggaagaccaacatcgcggaggccatagcccacactgtgcccttctacgggtgcgtaaactggaccaatgagaactttcccttcaacgactgtgtcgacaagatggtgatctggtgggaggaggggaagatgaccgccaaggtcgtggagtcggccaaagccattctcggaggaagcaaggtgcgcgtggaccagaaatgcaagtcctcggcccagatagacccgactcccgtgatcgtcacctccaacaccaacatgtgcgccgtgattgacgggaactcaacgaccttcgaacaccagcagccgttgcaagaccggatgttcaaatttgaactcacccgccgtctggatcatgactttgggaaggtcaccaagcaggaagtcaaagactttttccggtgggcaaaggatcacgtggttgaggtggagcatgaattctacgtcaaaaagggtggagccaagaaaagacccgcccccagtgacgcagatataagtgagcccaaacgggtgcgcgagtcagttgcgcagccatcgacgtcagacgcggaagcttcgatcaactacgcagacaggtaccaaaacaaatgttctcgtcacgtgggcatgaatctgatgctgtttccctgcagacaatgcgagagaatgaatcagaattcaaatatctgcttcactcacggacagaaagactgtttagagtgctttcccgtgtcagaatctcaacccgtttctgtcgtcaaaaaggcgtatcagaaactgtgctacattcatcatatcatgggaaaggtgccagacgcttgcactgcctgcgatctggtcaatgtggatttggatgactgcatctttgaacaataaatgatttaaatcaggtatggctgccgatggttatcttccagattggctcgaggacactctctctgaaggaataagacagtggtggaagctcaaacctggcccaccaccaccaaagcccgcagagcggcataaggacgacagcaggggtcttgtgcttcctgggtacaagtacctcggacccttcaacggactcgacaagggagagccggtcaacgaggcagacgccgcggccctcgagcacgacaaagcctacgaccggcagctcgacagcggagacaacccgtacctcaagtacaaccacgccgacgcggagtttcaggagcgccttaaagaagatacgtcttttgggggcaacctcggacgagcagtcttccaggcgaaaaagagggttcttgaacctctgggcctggttgaggaacctgttaagacggctccgggaaaaaagaggccggtagagcactctcctgtggagccagactcctcctcgggaaccggaaaggcgggccagcagcctgcaagaaaaagattgaattttggtcagactggagacgcagactcagtacctgacccccagcctctcggacagccaccagcagccccctctggtctgggaactaatacgatggctacaggcagtggcgcaccaatggcagacaataacgagggcgccgacggagtgggtaattcctcgggaaattggcattgcgattccacatggatgggcgacagagtcatcaccaccagcacccgaacctgggccctgcccacctacaacaaccacctctacaaacaaatttccagccaatcaggagcctcgaacgacaatcactactttggctacagcaccccttgggggtattttgacttcaacagattccactgccacttttcaccacgtgactggcaaagactcatcaacaacaactggggattccgacccaagagactcaacttcaagctctttaacattcaagtcaaagaggtcacgcagaatgacggtacgacgacgattgccaataaccttaccagcacggttcaggtgtttactgactcggagtaccagctcccgtacgtcctcggctcggcgcatcaaggatgcctcccgccgttcccagcagacgtcttcatggtgccacagtatggatacctcaccctgaacaacgggagtcaggcagtaggacgctcttcattttactgcctggagtactttccttctcagatgctgcgtaccggaaacaactttaccttcagctacacttttgaggacgttcctttccacagcagctacgctcacagccagagtctggaccgtctcatgaatcctctcatcgaccagtacctgtattacttgagcagaacaaacactccaagtggaaccaccacgcagtcaaggcttcagttttctcaggccggagcgagtgacattcgggaccagtctaggaactggcttcctggaccctgttaccgccagcagcgagtatcaaagacatctgcggataacaacaacagtgaatactcgtggactggagctaccaagtaccacctcaatggcagagactctctggtgaatccgggcccggccatggcaagccacaaggacgatgaagaaaagttttttcctcagagcggggttctcatctttgggaagcaaggctcagagaaaacaaatgtggacattgaaaaggtcatgattacagacgaagaggaaatcaggacaaccaatcccgtggctacggagcagtatggttctgtatctaccaacctccagagaggcaacagacaagcagctaccgcagatgtcaacacacaaggcgttcttccaggcatggtctggcaggacagagatgtgtaccttcaggggcccatctgggcaaagattccacacacggacggacattttcacccctctcccctcatgggtggattcggacttaaacaccctcctccacagattctcatcaagaacaccccggtacctgcgaatccttcgaccaccttcagtgcggcaaagtttgcttccttcatcacacagtactccacgggacaggtcagcgtggagatcgagtgggagctgcagaaggaaaacagcaaacgctggaatcccgaaattcagtacacttccaactacaacaagtctgttaatgtggactttactgtggacactaatggcgtgtattcagagcctcgccccattggcaccagatacctgactcgtaatctgtaattgcttgttaatcaataaaccgtttaattcgtttcagttgaactttggtctctgcgtatttctttcttatctagtttccatggctacgtagataagtagcatggcgggttaatcattaactacaatcagtgagcgagcgagcgcgcagcgatttcggggaaatgtgtaaactcgcaggtggcactta

SEQ ID NO: 8 - protein, 621 aa, adeno-associated virus 2
MPGFYEIVIKVPSDLDEHLPGISDSFVNWVAEKEWELPPDSDMDLNLIEQAPLTVAEKLQRDFLTEWRRVSKAPEALFFVQFEKGESYFHMHVLVETTGVKSMVLGRFLSQIREKLIQRIYRGIEPTLPNWFAVTKTRNGAGGGNKVVDECYIPNYLLPKTQPELQWAWTNMEQYLSACLNLTERKRLVAQHLTHVSQTQEQNKENQNPNSDAPVIRSKTSARYMELVGWLVDKGITSEKQWIQEDQASYISFNAASNSRSQIKAALDNAGKIMSLTKTAPDYLVGQQPVEDISSNRIYKILELNGYDPQYAASVFLGWATKKFGKRNTIWLFGPATTGKTNIAEAIAHTVPFYGCVNWTNENFPFNDCVDKMVIWWEEGKMTAKVVESAKAILGGSKVRVDQKCKSSAQIDPTPVIVTSNTNMCAVIDGNSTTFEHQQPLQDRMFKFELTRRLDHDFGKVTKQEVKDFFRWAKDHVVEVEHEFYVKKGGAKKRPAPSDADISEPKRVRESVAQPSTSDAEASINYADRYQNKCSRHVGMNLMLFPCRQCERMNQNSNICFTHGQKDCLECFPVSESQPVSVVKKAYQKLCYIHHIMGKVPDACTACDLVNVDLDDCIFEQ

SEQ ID NO: 9 - protein, 536 aa, adeno-associated virus 2
MPGFYEIVIKVPSDLDEHLPGISDSFVNWVAEKEWELPPDSDMDLNLIEQAPLTVAEKLQRDFLTEWRRVSKAPEALFFVQFEKGESYFHMHVLVETTGVKSMVLGRFLSQIREKLIQRIYRGIEPTLPNWFAVTKTRNGAGGGNKVVDECYIPNYLLPKTQPELQWAWTNMEQYLSACLNLTERKRLVAQHLTHVSQTQEQNKENQNPNSDAPVIRSKTSARYMELVGWLVDKGITSEKQWIQEDQASYISFNAASNSRSQIKAALDNAGKIMSLTKTAPDYLVGQQPVEDISSNRIYKILELNGYDPQYAASVFLGWATKKFGKRNTIWLFGPATTGKTNIAEAIAHTVPFYGCVNWTNENFPFNDCVDKMVIWWEEGKMTAKVVESAKAILGGSKVRVDQKCKSSAQIDPTPVIVTSNTNMCAVIDGNSTTFEHQQPLQDRMFKFELTRRLDHDFGKVTKQEVKDFFRWAKDHVVEVEHEFYVKKGGAKKRPAPSDADISEPKRVRESVAQPSTSDAEASINYADRLARGHSL

SEQ ID NO: 10 - protein, 397 aa, adeno-associated virus 2
MELVGWLVDKGITSEKQWIQEDQASYISFNAASNSRSQIKAALDNAGKIMSLTKTAPDYLVGQQPVEDISSNRIYKILELNGYDPQYAASVFLGWATKKFGKRNTIWLFGPATTGKTNIAEAIAHTVPFYGCVNWTNENFPFNDCVDKMVIWWEEGKMTAKVVESAKAILGGSKVRVDQKCKSSAQIDPTPVIVTSNTNMCAVIDGNSTTFEHQQPLQDRMFKFELTRRLDHDFGKVTKQEVKDFFRWAKDHVVEVEHEFYVKKGGAKKRPAPSDADISEPKRVRESVAQPSTSDAEASINYADRYQNKCSRHVGMNLMLFPCRQCERMNQNSNICFTHGQKDCLECFPVSESQPVSVVKKAYQKLCYIHHIMGKVPDACTACDLVNVDLDDCIFEQ

SEQ ID NO: 11 - protein, 312 aa, adeno-associated virus 2
MELVGWLVDKGITSEKQWIQEDQASYISFNAASNSRSQIKAALDNAGKIMSLTKTAPDYLVGQQPVEDISSNRIYKILELNGYDPQYAASVFLGWATKKFGKRNTIWLFGPATTGKTNIAEAIAHTVPFYGCVNWTNENFPFNDCVDKMVIWWEEGKMTAKVVESAKAILGGSKVRVDQKCKSSAQIDPTPVIVTSNTNMCAVIDGNSTTFEHQQPLQDRMFKFELTRRLDHDFGKVTKQEVKDFFRWAKDHVVEVEHEFYVKKGGAKKRPAPSDADISEPKRVRESVAQPSTSDAEASINYADRLARGHSL

SEQ ID NO: 12 - protein, 735 aa, adeno-associated virus 2 [sequence omitted]

SEQ ID NO: 13 - protein, 598 aa, adeno-associated virus 2
MAPGKKRPVEHSPVEPDSSSGTGKAGQQPARKRLNFGQTGDADSVPDPQPLGQPPAAPSGLGTNTMATGSGAPMADNNEGADGVGNSSGNWHCDSTWMGDRVITTSTRTWALPTYNNHLYKQISSQSGASNDNHYFGYSTPWGYFDFNRFHCHFSPRDWQRLINNNWGFRPKRLNFKLFNIQVKEVTQNDGTTTIANNLTSTVQVFTDSEYQLPYVLGSAHQGCLPPFPADVFMVPQYGYLTLNNGSQAVGRSSFYCLEYFPSQMLRTGNNFTFSYTFEDVPFHSSYAHSQSLDRLMNPLIDQYLYYLSRTNTPSGTTTQSRLQFSQAGASDIRDQSRNWLPGPCYRQQRVSKTSADNNNSEYSWTGATKYHLNGRDSLVNPGPAMASHKDDEEKFFPQSGVLIFGKQGSEKTNVDIEKVMITDEEEIRTTNPVATEQYGSVSTNLQRGNRQAATADVNTQGVLPGMVWQDRDVYLQGPIWAKIPHTDGHFHPSPLMGGFGLKHPPPQILIKNTPVPANPSTTFSAAKFASFITQYSTGQVSVEIEWELQKENSKRWNPEIQYTSNYNKSVNVDFTVDTNGVYSEPRPIGTRYLTRNL

SEQ ID NO: 14 - protein, 533 aa, adeno-associated virus 2
MATGSGAPMADNNEGADGVGNSSGNWHCDSTWMGDRVITTSTRTWALPTYNNHLYKQISSQSGASNDNHYFGYSTPWGYFDFNRFHCHFSPRDWQRLINNNWGFRPKRLNFKLFNIQVKEVTQNDGTTTIANNLTSTVQVFTDSEYQLPYVLGSAHQGCLPPFPADVFMVPQYGYLTLNNGSQAVGRSSFYCLEYFPSQMLRTGNNFTFSYTFEDVPFHSSYAHSQSLDRLMNPLIDQYLYYLSRTNTPSGTTTQSRLQFSQAGASDIRDQSRNWLPGPCYRQQRVSKTSADNNNSEYSWTGATKYHLNGRDSLVNPGPAMASHKDDEEKFFPQSGVLIFGKQGSEKTNVDIEKVMITDEEEIRTTNPVATEQYGSVSTNLQRGNRQAATADVNTQGVLPGMVWQDRDVYLQGPIWAKIPHTDGHFHPSPLMGGFGLKHPPPQILIKNTPVPANPSTTFSAAKFASFITQYSTGQVSVEIEWELQKENSKRWNPEIQYTSNYNKSVNVDFTVDTNGVYSEPRPIGTRYLTRNL

SEQ ID NO: 15 - protein, 204 aa, adeno-associated virus 2
METQTQYLTPSLSDSHQQPPLVWELIRWLQAVAHQWQTITRAPTEWVIPREIGIAIPHGWATESSPPAPEPGPCPPTTTTSTNKFPANQEPRTTITTLATAPLGGILTSTDSTATFHHVTGKDSSTTTGDSDPRDSTSSSLTFKSKRSRRMTVRRRLPITLPARFRCLLTRSTSSRTSSARRIKDASRRSQQTSSWCHSMDTSP

SEQ ID NO: 16 - protein, 155 aa, adeno-associated virus 2
MVLYLPTSREATDKQLPQMSTHKAFFQAWSGRTEMCTFRGPSGQRFHTRTDIFTPLPSWVDSDLNTLLHRFSSRTPRYLRILRPPSVRQSLLPSSHSTPRDRSAWRSSGSCRRKTANAGIPKFSTLPTTTSLLMWTLLWTLMACIQSLAPLAPDT

SEQ ID NO: 17 - protein, 265 aa, synthetic construct
MVSKGEELFTGVVPILVELDGDVNGHKFSVSGEGEGDATYGKLTLKFICTTGKLPVPWPTLVTTLTYGVQCFSRYPDHMKQHDFFKSAMPEGYVQERTIFFKDDGNYKTRAEVKFEGDTLVNRIELKGIDFKEDGNILGHKLEYNYNSHNVYIMADKQKNGIKVNFKIRHNIEDGSVQLADHYQQNTPIGDGPVLLPDNHYLSTQSALSKDPNEKRDHMVLLEFVTAAGITLGMDELYKSGLRSRAQASNSAVDGTAGPGSTGSR

SEQ ID NO: 18 - DNA, 22 bp, synthetic construct
  source 1..22: mol_type = other DNA
cagtgagcgagcgagcgcgcag